European Patent Application EP 4 184 515 A1, published May 24, 2023. Title: METHOD FOR DETERMINATION OF CELLULAR MRNA. Applicant: The Governing Council of the University of Toronto. Application EP, filed August 13, 2018. The sequence listing filed with the application follows.

SEQUENCE LISTING (31 sequences)

SEQ ID NO: 1 - DNA, 20 bp, synthetic construct
  misc_feature 1..20: note = Probe
  source 1..20: mol_type = other DNA
gataaggcttcctgccgcgc

SEQ ID NO: 2 - DNA, 20 bp, synthetic construct
  misc_feature 1..20: note = Probe
  source 1..20: mol_type = other DNA
caacgactggtcctcactca

SEQ ID NO: 3 - DNA, 45 bp, synthetic construct
  misc_feature 1..45: note = probe
  source 1..45: mol_type = other DNA
gcgcggcaggaagccttatcagttgtgagtgaggaccagtcgttg

SEQ ID NO: 4 - DNA, 45 bp, synthetic construct
  misc_feature 1..45: note = Ctrl-TMPRSS2/ERG oligonucleotide
  source 1..45: mol_type = other DNA
gttgctgaccaggagtgagtgttgactattccgaaggacggcgcg

SEQ ID NO: 5 - DNA, 20 bp, synthetic construct
  misc_feature 1..20: note = Probe
  source 1..20: mol_type = other DNA
gataaggcttcctgccgcgc

SEQ ID NO: 6 - DNA, 20 bp, synthetic construct
  misc_feature 1..20: note = Probe
  source 1..20: mol_type = other DNA
caacgactggtcctcactca

SEQ ID NO: 7 - DNA, 20 bp, synthetic construct
  misc_feature 1..20: note = Probe
  source 1..20: mol_type = other DNA
cagttcttgaatgtagagat

SEQ ID NO: 8 - DNA, 20 bp, synthetic construct
  misc_feature 1..20: note = Probe
  source 1..20: mol_type = other DNA
gcaggcgcagccctccaaga

SEQ ID NO: 9 - DNA, 20 bp, synthetic construct
  misc_feature 1..20: note = Probe
  source 1..20: mol_type = other DNA
tgctttcatgcacaggaatt

SEQ ID NO: 10 - DNA, 20 bp, synthetic construct
  misc_feature 1..20: note = Probe
  source 1..20: mol_type = other DNA
ctggaataatgctgaagagt

SEQ ID NO: 11 - DNA, 20 bp, synthetic construct
  misc_feature 1..20: note = Probe
  source 1..20: mol_type = other DNA
ctgatgaagagaagcatgtg

SEQ ID NO: 12 - DNA, 20 bp, synthetic construct
  misc_feature 1..20: note = Probe
  source 1..20: mol_type = other DNA
tgggagaagaatgagaggct

SEQ ID NO: 13 - DNA, 18 bp, synthetic construct
  misc_feature 1..18: note = LY2181308 antisense oligonucleotide
  source 1..18: mol_type = other DNA
tgtgctattctgtgaatt

SEQ ID NO: 14 - DNA, 17 bp, synthetic construct
  misc_feature 1..17: note = Primer
  source 1..17: mol_type = other DNA
caggaggcggaggcgga

SEQ ID NO: 15 - DNA, 21 bp, synthetic construct
  misc_feature 1..21: note = Primer
  source 1..21: mol_type = other DNA
ggcgttgtagctgggggtgag

SEQ ID NO: 16 - DNA, 23 bp, synthetic construct
  misc_feature 1..23: note = Primer
  source 1..23: mol_type = other DNA
ctttctcaaggaccaccgcatct

SEQ ID NO: 17 - DNA, 22 bp, synthetic construct
  misc_feature 1..22: note = Primer
  source 1..22: mol_type = other DNA
gcactttctccgcagtttcctc

SEQ ID NO: 18 - DNA, 21 bp, synthetic construct
  misc_feature 1..21: note = Primer
  source 1..21: mol_type = other DNA
ggaattcctgtgcatgaaagc

SEQ ID NO: 19 - DNA, 24 bp, synthetic construct
  misc_feature 1..24: note = Primer
  source 1..24: mol_type = other DNA
cgatcgagttccttgatgtagttc

SEQ ID NO: 20 - DNA, 24 bp, synthetic construct
  misc_feature 1..24: note = Primer
  source 1..24: mol_type = other DNA
cttgtcgtcttcggaaatgttatg

SEQ ID NO: 21 - DNA, 22 bp, synthetic construct
  misc_feature 1..22: note = Primer
  source 1..22: mol_type = other DNA
ctttcttcagggtctggtcatt

SEQ ID NO: 22 - DNA, 20 bp, synthetic construct
  misc_feature 1..20: note = Primer
  source 1..20: mol_type = other DNA
cggctgtttaacttcgcttc

SEQ ID NO: 23 - DNA, 20 bp, synthetic construct
  misc_feature 1..20: note = Primer
  source 1..20: mol_type = other DNA
cacacgccaagaaacagtga

SEQ ID NO: 24 - DNA, 20 bp, synthetic construct
  misc_feature 1..20: note = Primer
  source 1..20: mol_type = other DNA
gagtcaacggatttggtcgt

SEQ ID NO: 25 - DNA, 20 bp, synthetic construct
  misc_feature 1..20: note = Primer
  source 1..20: mol_type = other DNA
gacaagcttcccgttctcag

SEQ ID NO: 26 - DNA, 20 bp, synthetic construct
  misc_feature 1..20: note = Probe
  source 1..20: mol_type = other DNA
tgttcagaggtgactggatc

SEQ ID NO: 27 - DNA, 20 bp, synthetic construct
  misc_feature 1..20: note = Probe
  source 1..20: mol_type = other DNA
gccctcagcctgacatgtca

SEQ ID NO: 28 - DNA, 20 bp, synthetic construct
  misc_feature 1..20: note = Probe
  source 1..20: mol_type = other DNA
ctcagggacacagggcacgg

SEQ ID NO: 29 - DNA, 20 bp, synthetic construct
  misc_feature 1..20: note = Probe
  source 1..20: mol_type = other DNA
agacaatggtggcatactcc

SEQ ID NO: 30 - DNA, 20 bp, synthetic construct
  misc_feature 1..20: note = Probe
  source 1..20: mol_type = other DNA
tctgtagcaaggaggctgaa

SEQ ID NO: 31 - DNA, 20 bp, synthetic construct
  misc_feature 1..20: note = Probe
  source 1..20: mol_type = other DNA
ctgcttcttcagggcttctt